European Patent Application EP 4 726 033 A1, published April 15, 2026. Title: 신규한 아세토아세틸-CoA 리덕타아제 변이체 및 이의 용도. Applicant: 씨제이제일제당 (주). The sequence listing filed with the application follows.

SEQUENCE LISTING (82 sequences)

SEQ ID NO: 1 - protein, 246 aa, Cupriavidus necator
MTQRIAYVTGGMGGIGTAICQRLAKDGFRVVAGCGPNSPRREKWLEQQKALGFDFIASEGNVADWDSTKTAFDKVKSEVGEVDVLINNAGITRDVVFRKMTRADWDAVIDTNLTSLFNVTKQVIDGMADRGWGRIVNISSVNGQKGQFGQTNYSTAKAGLHGFTMALAQEVATKGVTVNTVSPGYIATDMVKAIRQDVLDKIVATIPVKRLGLPEEIASICAWLSSEESGFSTGADFSLNGGLHMG

SEQ ID NO: 2 - DNA, 741 bp, Cupriavidus necator
  source 1..741: mol_type = genomic DNA
atgactcagcgcattgcgtatgtgaccggcggcatgggtggtatcggaaccgccatttgccagcggctggccaaggatggctttcgtgtggtggccggttgcggccccaactcgccgcgccgcgaaaagtggctggagcagcagaaggccctgggcttcgatttcattgcctcggaaggcaatgtggctgactgggactcgaccaagaccgcattcgacaaggtcaagtccgaggtcggcgaggttgatgtgctgatcaacaacgccggtatcacccgcgacgtggtgttccgcaagatgacccgcgccgactgggatgcggtgatcgacaccaacctgacctcgctgttcaacgtcaccaagcaggtgatcgacggcatggccgaccgtggctggggccgcatcgtcaacatctcgtcggtgaacgggcagaagggccagttcggccagaccaactactccaccgccaaggccggcctgcatggcttcaccatggcactggcgcaggaagtggcgaccaagggcgtgaccgtcaacacggtctctccgggctatatcgccaccgacatggtcaaggcgatccgccaggacgtgctcgacaagatcgtcgcgacgatcccggtcaagcgcctgggcctgccggaagagatcgcctcgatctgcgcctggttgtcgtcggaggagtccggtttctcgaccggcgccgacttctcgctcaacggcggcctgcatatgggctga

SEQ ID NO: 3 - protein, 246 aa, synthetic construct
MTQRIAYVTGGMGGIGTAICQRLAKDGFRVVAGCAPNSPRREKWLEQQKALGFDFIASEGNVADWDSTKTAFDKVKSEVGEVDVLINNAGITRDVVFRKMTRADWDAVIDTNLTSLFNVTKQVIDGMADRGWGRIVNISSVNGQKGQFGQTNYSTAKAGLHGFTMALAQEVATKGVTVNTVSPGYIATDMVKAIRQDVLDKIVATIPVKRLGLPEEIASICAWLSSEESGFSTGADFSLNGGLHMG

SEQ ID NO: 4 - DNA, 50 bp, synthetic construct
  source 1..50: mol_type = other DNA
cggtacccggggatcctctagagaaccactatcaatatattcatgtcgaa

SEQ ID NO: 5 - DNA, 37 bp, synthetic construct
  source 1..37: mol_type = other DNA
caagcttgcatgcctgcaggtttgcctggcggcagta

SEQ ID NO: 6 - DNA, 39 bp, synthetic construct
  source 1..39: mol_type = other DNA
gcgtatgtgaccggcggcagcggtggtatcggaaccgcc

SEQ ID NO: 7 - DNA, 39 bp, synthetic construct
  source 1..39: mol_type = other DNA
ggcggttccgataccaccgctgccgccggtcacatacgc

SEQ ID NO: 8 - DNA, 40 bp, synthetic construct
  source 1..40: mol_type = other DNA
cgtgtggtggccggttgcgcccccaactcgccgcgccgcg

SEQ ID NO: 9 - DNA, 40 bp, synthetic construct
  source 1..40: mol_type = other DNA
cgcggcgcggcgagttgggggcgcaaccggccaccacacg

SEQ ID NO: 10 - DNA, 50 bp, synthetic construct
  source 1..50: mol_type = other DNA
gatttcattgcctcggaaggcgatgtggctgactgggactcgaccaagac

SEQ ID NO: 11 - DNA, 50 bp, synthetic construct
  source 1..50: mol_type = other DNA
gtcttggtcgagtcccagtcagccacatcgccttccgaggcaatgaaatc

SEQ ID NO: 12 - DNA, 48 bp, synthetic construct
  source 1..48: mol_type = other DNA
gatttcattgcctcggaaggcaatacggctgactgggactcgaccaag

SEQ ID NO: 13 - DNA, 48 bp, synthetic construct
  source 1..48: mol_type = other DNA
cttggtcgagtcccagtcagccgtattgccttccgaggcaatgaaatc

SEQ ID NO: 14 - DNA, 42 bp, synthetic construct
  source 1..42: mol_type = other DNA
gaacgggcagaagggccagtacggccagaccaactactccac

SEQ ID NO: 15 - DNA, 42 bp, synthetic construct
  source 1..42: mol_type = other DNA
gtggagtagttggtctggccgtactggcccttctgcccgttc

SEQ ID NO: 16 - DNA, 41 bp, synthetic construct
  source 1..41: mol_type = other DNA
ccaccgacatggtcaaggcgatgcgccaggacgtgctcgac

SEQ ID NO: 17 - DNA, 41 bp, synthetic construct
  source 1..41: mol_type = other DNA
gtcgagcacgtcctggcgcatcgccttgaccatgtcggtgg

SEQ ID NO: 18 - DNA, 43 bp, synthetic construct
  source 1..43: mol_type = other DNA
ggtcaaggcgatccgccaggacacgctcgacaagatcgtcgcg

SEQ ID NO: 19 - DNA, 43 bp, synthetic construct
  source 1..43: mol_type = other DNA
cgcgacgatcttgtcgagcgtgtcctggcggatcgccttgacc

SEQ ID NO: 20 - DNA, 40 bp, synthetic construct
  source 1..40: mol_type = other DNA
cgcgaaaagtggctggagctgcagaaggccctgggcttcg

SEQ ID NO: 21 - DNA, 40 bp, synthetic construct
  source 1..40: mol_type = other DNA
cgaagcccagggccttctgcagctccagccacttttcgcg

SEQ ID NO: 22 - DNA, 41 bp, synthetic construct
  source 1..41: mol_type = other DNA
ctggcgcaggaagtggcgtccaagggcgtgaccgtcaacac

SEQ ID NO: 23 - DNA, 41 bp, synthetic construct
  source 1..41: mol_type = other DNA
gtgttgacggtcacgcccttggacgccacttcctgcgccag

SEQ ID NO: 24 - DNA, 40 bp, synthetic construct
  source 1..40: mol_type = other DNA
cgtgtggtggccggttgccaccccaactcgccgcgccgcg

SEQ ID NO: 25 - DNA, 40 bp, synthetic construct
  source 1..40: mol_type = other DNA
cgcggcgcggcgagttggggtggcaaccggccaccacacg

SEQ ID NO: 26 - DNA, 40 bp, synthetic construct
  source 1..40: mol_type = other DNA
cgtgtggtggccggttgcgtccccaactcgccgcgccgcg

SEQ ID NO: 27 - DNA, 40 bp, synthetic construct
  source 1..40: mol_type = other DNA
cgcggcgcggcgagttggggacgcaaccggccaccacacg

SEQ ID NO: 28 - DNA, 40 bp, synthetic construct
  source 1..40: mol_type = other DNA
cgtgtggtggccggttgctcccccaactcgccgcgccgcg

SEQ ID NO: 29 - DNA, 40 bp, synthetic construct
  source 1..40: mol_type = other DNA
cgcggcgcggcgagttgggggagcaaccggccaccacacg

SEQ ID NO: 30 - DNA, 36 bp, synthetic construct
  source 1..36: mol_type = other DNA
cggtcgtcgcgggttgcgccccgaactctccgcgcc

SEQ ID NO: 31 - DNA, 36 bp, synthetic construct
  source 1..36: mol_type = other DNA
ggcgcggagagttcggggcgcaacccgcgacgaccg

SEQ ID NO: 32 - DNA, 40 bp, synthetic construct
  source 1..40: mol_type = other DNA
ctgcaccgtcgtggcgaactgcgctccgtccgaggcggcc

SEQ ID NO: 33 - DNA, 40 bp, synthetic construct
  source 1..40: mol_type = other DNA
ggccgcctcggacggagcgcagttcgccacgacggtgcag

SEQ ID NO: 34 - DNA, 41 bp, synthetic construct
  source 1..41: mol_type = other DNA
caaagtcatcgtcggatgcgccccacaatccaaacgcaaag

SEQ ID NO: 35 - DNA, 41 bp, synthetic construct
  source 1..41: mol_type = other DNA
ctttgcgtttggattgtggggcgcatccgacgatgactttg

SEQ ID NO: 36 - DNA, 40 bp, synthetic construct
  source 1..40: mol_type = other DNA
ggtcatcgccggctgcgctccgagccgcgactaccagaag

SEQ ID NO: 37 - DNA, 40 bp, synthetic construct
  source 1..40: mol_type = other DNA
cttctggtagtcgcggctcggagcgcagccggcgatgacc

SEQ ID NO: 38 - DNA, 39 bp, synthetic construct
  source 1..39: mol_type = other DNA
ccgcgttgcagtgacctgtgcccccacgaatcacgattg

SEQ ID NO: 39 - DNA, 39 bp, synthetic construct
  source 1..39: mol_type = other DNA
caatcgtgattcgtgggggcacaggtcactgcaacgcgg

SEQ ID NO: 40 - DNA, 41 bp, synthetic construct
  source 1..41: mol_type = other DNA
ctacgcggtcgtcgtgacgcatgcgccgggcaacgcgaagg

SEQ ID NO: 41 - DNA, 41 bp, synthetic construct
  source 1..41: mol_type = other DNA
ccttcgcgttgcccggcgcatgcgtcacgacgaccgcgtag

SEQ ID NO: 42 - DNA, 40 bp, synthetic construct
  source 1..40: mol_type = other DNA
cacaaggtggttgccgcctacgctccggagttcgacaagc

SEQ ID NO: 43 - DNA, 40 bp, synthetic construct
  source 1..40: mol_type = other DNA
gcttgtcgaactccggagcgtaggcggcaaccaccttgtg

SEQ ID NO: 44 - DNA, 49 bp, synthetic construct
  source 1..49: mol_type = other DNA
ctcacgatgctcgcgtattgagatatcaaccactatcaatatattcatg

SEQ ID NO: 45 - DNA, 47 bp, synthetic construct
  source 1..47: mol_type = other DNA
cgaaagtttgaggcgtaaaaagcgatatctttgcctggcggcagtag

SEQ ID NO: 46 - DNA, 40 bp, synthetic construct
  source 1..40: mol_type = other DNA
ccgggctgcaggaattcgatacgaaacacgcgttcattga

SEQ ID NO: 47 - DNA, 49 bp, synthetic construct
  source 1..49: mol_type = other DNA
catgaatatattgatagtggttgatatctcaatacgcgagcatcgtgag

SEQ ID NO: 48 - DNA, 47 bp, synthetic construct
  source 1..47: mol_type = other DNA
ctactgccgccaggcaaagatatcgctttttacgcctcaaactttcg

SEQ ID NO: 49 - DNA, 40 bp, synthetic construct
  source 1..40: mol_type = other DNA
gctaggtcgactagcgtgatgcacacgccgatgcttttga

SEQ ID NO: 50 - protein, 246 aa, Pseudomonas putida
MTKRIAYVTGGMGGIGTSICQRLHKDGYTVVAGCGPNSPRRVKWLEEQKANGYDFIASEGNVGDWESTKNAFDKVKAEVGEVDILVNNAGITRDVVFRKMTHEDWTAVIDTNLTSLFNVTKQVVDGMVERGFGRIINISSVNGQKGQFGQTNYSTAKAGIHGFTMALAQEVATKGVTVNTVSPGYIGTDMVKAIRPEVLEKIVATIPVRRLGRPDEIGSIVSWLASEESGFSTGADFSLNGGLHMG

SEQ ID NO: 51 - protein, 245 aa, Alcaligenes sp.
MTQKLAYVTGGMGGIGTSMCQRLHKDGFKVIAGCGPSRDYQKWLDEQKALGYTFYASVGNVADWDSTVVAFEKVKAEHGTVDVLVNNAGITRDGQFRKMSKADWQAVMSTNLDSMFNVTKQVIDGMLDKGWGRIINISSVNGEKGQFGQTNYSAAKAGMHGFTMALAQEVAAKGVTVNTVSPGYIATDMVKAIRQDVLDKIVSTIPIKRLGTPEEIASIVAWLAGDESGFTTGADFSCNGGLHMG

SEQ ID NO: 52 - protein, 246 aa, Allochromatium vinosum
MARIALVTGGIGGIGTSICTRLAKDGCTVVANCHPSEAAAAEEWKQARAAEGFDIAVFTADVSSFDDSARMVREITEQVGPIDILVNCAGITRDKTFKKMEQAHWEAVINVNLNSVFNVTRQVWDGMLERGFGRIINISSVNGQRGQFGQANYSAAKAGMHGFTMALAQEGASKGVTVNTISPGYVETAMTLAMNDDVRNSIISGIPMRRMAQPDEIAAAIAFLAGDESGYMTGANLPVNGGLFMH

SEQ ID NO: 53 - protein, 247 aa, Azotobacter beijerinckii
MSNQRIAFVTGGMGGIGTSISQRLHKEGFTVIVGCTPQSKRKDGWLASQRDSGFSFEACEHDVTDWESTQRAFAELRERVGTIDVLVNNAGITRDASFRKLTPENWNAVISTNLNGMFNATKQVIEDMLGKGWGRIINISSINGQRGQFGQTNYSAAKAGIHGFTMALAREVASKGVTVNTISPGYILTEMTGAMRPEVLEQIAAGIPVGRLGKPEEIASMVAWLASDEAAYATGADFSINGGLNMQ

SEQ ID NO: 54 - protein, 247 aa, Pandoraea sp.
MTTRIALVTGGMGGLGEAISLRLADAGYRVAVTCSPQNHDCEGWVERMRATGREFAAYRVDVADFASCEACAKAVESDTGPVDILINNAGITRDATMRKMTSEDWQSVLRTNLDSVFNMTRPIFGGMVARGWGRIVNISSVNGSRGAFGQANYAAAKAGMHGFTKSLALEVAKAGVTVNTISPGYLATKMVTAVPADVLESRILPQIPVGRLGRPDEVAALVAFLASEDAGFITGSNLAINGGMHME

SEQ ID NO: 55 - protein, 247 aa, unidentified
MTKRIALVTGGMGGLGEAISVRLHDAAYDVVVTHTPGNPNVHNWLATMEAAGRNFRAYALDVADYDACQTTMAKILAEVGQVDILVNNAGITRDMAFKKMDKVNWDAVIRTNLDSVFNVTKPLCEGMVERGWGRIINISSINGSKGAFGQTNYAAAKAGMHGFTKSLALEVARKGVTVNTISPGYLATKMVTAVPQEIMDTKILPQIPVGRLGKPEEVAALVAYLCSEDAAYVTGSNIAINGGQHMQ

SEQ ID NO: 56 - protein, 247 aa, unidentified
MTQRVALVTGAMGGIGTAICQELAKAGHKVVAAYHPEFDKPEEWTKAMAEAGFNDFICVAGDVSDYDSCVALTAEAEAKAGPIDILVNNAGITRDKMFARMELAQWNAVISTNLNSLFNMTKQVSSKMAERGWGRIINISSLNGLKGQAGQTNYSAAKAGVIGFTKALAAELAAKGVTVNAICPGYVATPMVMAIKPEILQGIIDTVPMKRLAKPEEIGGACAYLASDIAGFMTGSTMNICGGLYYQ

SEQ ID NO: 57 - protein, 246 aa, synthetic construct
MTKRIAYVTGGMGGIGTSICQRLHKDGYTVVAGCAPNSPRRVKWLEEQKANGYDFIASEGNVGDWESTKNAFDKVKAEVGEVDILVNNAGITRDVVFRKMTHEDWTAVIDTNLTSLFNVTKQVVDGMVERGFGRIINISSVNGQKGQFGQTNYSTAKAGIHGFTMALAQEVATKGVTVNTVSPGYIGTDMVKAIRPEVLEKIVATIPVRRLGRPDEIGSIVSWLASEESGFSTGADFSLNGGLHMG

SEQ ID NO: 58 - protein, 245 aa, synthetic construct
MTQKLAYVTGGMGGIGTSMCQRLHKDGFKVIAGCAPSRDYQKWLDEQKALGYTFYASVGNVADWDSTVVAFEKVKAEHGTVDVLVNNAGITRDGQFRKMSKADWQAVMSTNLDSMFNVTKQVIDGMLDKGWGRIINISSVNGEKGQFGQTNYSAAKAGMHGFTMALAQEVAAKGVTVNTVSPGYIATDMVKAIRQDVLDKIVSTIPIKRLGTPEEIASIVAWLAGDESGFTTGADFSCNGGLHMG

SEQ ID NO: 59 - protein, 246 aa, synthetic construct
MARIALVTGGIGGIGTSICTRLAKDGCTVVANCAPSEAAAAEEWKQARAAEGFDIAVFTADVSSFDDSARMVREITEQVGPIDILVNCAGITRDKTFKKMEQAHWEAVINVNLNSVFNVTRQVWDGMLERGFGRIINISSVNGQRGQFGQANYSAAKAGMHGFTMALAQEGASKGVTVNTISPGYVETAMTLAMNDDVRNSIISGIPMRRMAQPDEIAAAIAFLAGDESGYMTGANLPVNGGLFMH

SEQ ID NO: 60 - protein, 247 aa, synthetic construct
MSNQRIAFVTGGMGGIGTSISQRLHKEGFTVIVGCAPQSKRKDGWLASQRDSGFSFEACEHDVTDWESTQRAFAELRERVGTIDVLVNNAGITRDASFRKLTPENWNAVISTNLNGMFNATKQVIEDMLGKGWGRIINISSINGQRGQFGQTNYSAAKAGIHGFTMALAREVASKGVTVNTISPGYILTEMTGAMRPEVLEQIAAGIPVGRLGKPEEIASMVAWLASDEAAYATGADFSINGGLNMQ

SEQ ID NO: 61 - protein, 247 aa, synthetic construct
MTTRIALVTGGMGGLGEAISLRLADAGYRVAVTCAPQNHDCEGWVERMRATGREFAAYRVDVADFASCEACAKAVESDTGPVDILINNAGITRDATMRKMTSEDWQSVLRTNLDSVFNMTRPIFGGMVARGWGRIVNISSVNGSRGAFGQANYAAAKAGMHGFTKSLALEVAKAGVTVNTISPGYLATKMVTAVPADVLESRILPQIPVGRLGRPDEVAALVAFLASEDAGFITGSNLAINGGMHME

SEQ ID NO: 62 - protein, 247 aa, synthetic construct
MTKRIALVTGGMGGLGEAISVRLHDAAYDVVVTHAPGNPNVHNWLATMEAAGRNFRAYALDVADYDACQTTMAKILAEVGQVDILVNNAGITRDMAFKKMDKVNWDAVIRTNLDSVFNVTKPLCEGMVERGWGRIINISSINGSKGAFGQTNYAAAKAGMHGFTKSLALEVARKGVTVNTISPGYLATKMVTAVPQEIMDTKILPQIPVGRLGKPEEVAALVAYLCSEDAAYVTGSNIAINGGQHMQ

SEQ ID NO: 63 - protein, 247 aa, synthetic construct
MTQRVALVTGAMGGIGTAICQELAKAGHKVVAAYAPEFDKPEEWTKAMAEAGFNDFICVAGDVSDYDSCVALTAEAEAKAGPIDILVNNAGITRDKMFARMELAQWNAVISTNLNSLFNMTKQVSSKMAERGWGRIINISSLNGLKGQAGQTNYSAAKAGVIGFTKALAAELAAKGVTVNAICPGYVATPMVMAIKPEILQGIIDTVPMKRLAKPEEIGGACAYLASDIAGFMTGSTMNICGGLYYQ

SEQ ID NO: 64 - DNA, 741 bp, Pseudomonas putida
  source 1..741: mol_type = genomic DNA
atgacgaaacgcatagcgtacgtgacgggcggcatgggcggcattggcacaagcatctgccagcgtctgcataaggacggctatacggtcgtcgcgggttgcggcccgaactctccgcgccgtgtcaaatggctcgaggaacagaaggcgaacggctatgacttcatcgcgtccgagggcaacgtcggcgactgggagtccaccaagaacgccttcgacaaggtgaaagccgaagtcggcgaagtcgacatcctggtgaacaacgcgggcatcacgcgcgacgtcgtgttccgcaagatgacgcacgaggactggacggccgtcatccacaccaacctgacgagcctcttcaacgtgaccaagcaggtggtccacggcatggtggagcgcggtttcgggcggatcatcaacatttcgtcggtgaacggccacaaagggcagttcggccagaccaactactctacggcgaaagccggcatccacggcttcacgatggcgctcgcgcaggaagtggcgaccaagggcgtgacggtcaacaccgtgtcgccaggctatatcggcacggacatggtcaaggcgatccgccccgaggtgctggagaagatcgtcgcgacgattccggtgcgccgtctcggccgcccggacgagatcggctcgatcgtgtcgtggctggcatcggaggaatcgggcttctcgaccggtgcggacttctcgctcaacggcgggctgcacatgggctga

SEQ ID NO: 65 - DNA, 738 bp, Alcaligenes sp.
  source 1..738: mol_type = genomic DNA
atgactcaaaaactcgcttacgtgacgggcggcatgggcggcatcggtacttcgatgtgccaacgcctgcacaaggacggcttcaaggtcatcgccggctgcggtccgagccgcgactaccagaagtggctggacgagcagaaggccctgggctacacgttctacgcctcggtgggcaacgtggccgactgggactccaccgtcgtcgccttcgagaaggtcaaggccgagcacggcacggtggacgtgctggtgaacaacgccggcatcacgcgtgacggccagttccgcaagatgagcaaggccgattggcaggccgtgatgtccaccaacctggacagcatgttcaacgtcaccaagcaggtgatcgacggcatgctggacaagggctggggccgcatcatcaacatctcctcggtcaacggcgagaagggccagttcggccagaccaactactccgccgccaaggccggcatgcacggcttcaccatggccctggcgcaggaagtggctgccaagggcgtgacggtcaacaccgtgagccccggctacatcgccaccgacatggtcaaggccatccgccaggacgtgctggacaagatcgtctccaccattcccatcaagcgcctgggcaccccggaggaaatcgcctccatcgtggcctggctggcgggcgacgaatccggcttcaccaccggtgccgacttcagctgcaacggcggcctgcacatgggctga

SEQ ID NO: 66 - DNA, 741 bp, Allochromatium vinosum
  source 1..741: mol_type = genomic DNA
atggctcgtatcgcactcgtcaccggcggcatcggcggcatcggcacttcgatctgcacacgcctggcaaaggatggctgcaccgtcgtggcgaactgccatccgtccgaggcggccgccgccgaagagtggaagcaggcccgtgccgccgaggggttcgacatcgccgtctttaccgctgacgtgtcctcgttcgacgacagcgcgcgcatggttcgcgagatcacagagcaggtcggtcccatcgacatcctggtcaactgtgccggcatcacccgcgacaagaccttcaagaagatggagcaggcgcactgggaggccgtgatcaacgtcaacctcaacagcgtcttcaacgtcacccgtcaggtgtgggacgggatgctggagcgcggcttcgggcgtatcatcaacatctcgtcggtcaacggtcagcgcggccagttcggtcaggccaactattccgccgccaaggccggtatgcacggcttcaccatggctctggctcaggagggtgcgtccaagggcgtgaccgtcaacaccatctcgcccggctatgtcgagacggccatgaccctggcgatgaacgacgatgtgcgcaacagcatcatcagcggtattccgatgcgtcgcatggctcagcctgatgagatcgccgccgccatcgctttcctggccggcgacgagagcggttatatgacgggcgccaatctgccggtcaacggcggtctgttcatgcattga

SEQ ID NO: 67 - DNA, 744 bp, Azotobacter beijerinckii
  source 1..744: mol_type = genomic DNA
atgagcaatcaacgaattgcattcgtaacgggcggcatgggtggaatcgggacctcaatcagtcagcgcctttacaaggaaaatttcaaagtcatcgtcggatgcaccccacaatccaaacgcaaagatggctggctctccgcccagcgcgatagcggtttcagcttcgaagcctgtgaacatgacgtcaccgattgggaaagcacccagcgtgccttcgccgaactgcgcgaacgcgtcggcacaatcgatgtgctagtaaacaatgctggcattacccgcgacgccagcttccgcaagctcactccggaaaactggagtgcagtgatcaacaccaacctcaacggcatgttcaacaccaccaaacaggtcattgaagacatgctcggcaagggctggggccgcatcatcaacatctcctccatcaacggccagcgcggccagttcggccagaccaactactccgcggccaaagccggtattcatggcttcaccatggccctggcccgcgaagtggccagcaagggcgtgaccgtcaacacgatttcccctggctacatcctcaccgaaatgactggagccatgcgcccggaagttctcgaacagatcgctgccggcattccggtcggtcgccttggacagcccgaggaaatcgccagcatggttgcctggctggcctctgatgaggctgcctatgccactggcgccgacttctccatcaacggcggtctgaacatgcaatga

SEQ ID NO: 68 - DNA, 744 bp, Pandoraea sp.
  source 1..744: mol_type = genomic DNA
atgacaacacgaatcgctttggtgactggcggcatgggtgggctgggcgaggccatcagcctgcgtcttgccgatgccggataccgcgttgcagtgacctgttcccccacgaatcacgattgcgaaggctgggtcgagcgcatgcgcgagaccggtcgtgaattcgctgcctatcgtgtcgacgttgccgacttcgcgtcatgcgaggcctgcgcgagggcggtggaatccgacacggggccggtggacattctcatcaacaatgcggggatcacgcgcgacgccacgatgcgcaagatgacggccgaggactggcagtcggtattgcgcacgaatctggacagcgttttcaacatgacccgcccgctcttcgggggcatggtggcgcgtggttggggacgcatcatcaacgtcgcgtcggtcaacggcagtcgcggcgctttcgggcaggcgaactatgcggcgtcgaaggcgggcatgcacggattcaccaaatccctcgccctggaagtcgccaaatcgggggtcaccgtcaacaccatctcgccggggtacctcgcgacgaagatggtcacagcggtgccaaaggaagtgctcgaatcgcgcattcttccgcaaattccggtcggtcgcctcggacggcccgacgaggtggccgcgctcgtcgcattcctcgtatctgacgacgccgctttcatcaccggaagcaacctcgccatcaacggcggcatgcacatggagtag

SEQ ID NO: 69 - DNA, 744 bp, unidentified
  source 1..744: mol_type = genomic DNA
atgactaagcgaatcgcactggtgaccggcggcatgggcggactcggcgaggcagtcgccatcaagctgcacgacgcaggctacgcggtcgtcgtgacgcattcgccgggcaacgcgaaggccggcgaatggctcgcgagcatggatcgccagggccgcaacttccgcgcgtatccggtcgacgtcgccgattacgattccgcccagcactgcgtcgcgaagatccaggccgaagtcggcccgatcgatatcctcgtgaacaacgccggcatcacgcaggacacgaccttcaagaagatgaccaaggtgaactgggacgcggtgctgcgcaccaatctcgattcggtcttcaacatgaccaagccggtttgcgaagagatggtgtcgcgcggctggggtcgcatcatcaacatttcgtcggtgaatggatcgaaaggccagatcggtcagacgaactattcggcggcgaaggcgggcatgcacggcttcacgaagtcgctcgcgctcgaagtcgcgaagaagggcgtgaccgtgaacacgatctcgccgggctatctcgcgaccaagatggtgaccgcgattccgcaggagattctcgacacgaagattcttccgcagattccggcgggacgtctcggcaagcccgaggaagtcgcggcgctcgtcgcgttcctgtgctcggacgatgcgggtttcgtcaccggttcgaacatcgcgatcaacggcggccagcacatgagctga

SEQ ID NO: 70 - DNA, 744 bp, unidentified
  source 1..744: mol_type = genomic DNA
atgacgcaacgtgttgctttggttacaggtgctatgggtggaatcggaacggctgtttgccaggaactggccaaggccggccacaaggtggttgccgcctaccatccggagttcgacaagccggaagagtggacaaaggccatggctgaagccggtttcaacgatttcatctgtgtcgctggcgatgtctccgactatgactcctgcgtcgctcttaccgcggaggcggaagccaaggtaggtccgatcgacattctggtcaacaatgccggcatcacacgtgacaagatgttcgcgcggatggagctggcgcagtggaatgccgtgatttcaaccaacctcaatagcctcttcaacatgaccaagcaggtctcatcgaagatggccgagcgcggctggggcaggatcatcaacatctcctcggttaatggcctccgtggccaagctggtcagaccaattactccgccgccaaagcgggcgtgattggctttaccaaggcgctggccgccgagctggccgccaagaacgtgacggtcaacgccatttgccctggctatgtagccaccccaatggtgatggcgatcaagccggaggtcctgcagagcatcatcgatacggtgccgatgaagcgtctggcgaagccggaagaaatcgggggtgcgtgtgcctaccttgcttcggacattgccggcttcatgacgggttcgacgatgaacatctgtggcggcctctactatcagtag

SEQ ID NO: 71 - DNA, 741 bp, synthetic construct
  source 1..741: mol_type = other DNA
atgactcagcgcattgcgtatgtgaccggcggcatgggtggtatcggaaccgccatttgccagcggctggccaaggatggctttcgtgtggtggccggttgcgcccccaactcgccgcgccgcgaaaagtggctggagcagcagaaggccctgggcttcgatttcattgcctcggaaggcaatgtggctgactgggactcgaccaagaccgcattcgacaaggtcaagtccgaggtcggcgaggttgatgtgctgatcaacaacgccggtatcacccgcgacgtggtgttccgcaagatgacccgcgccgactgggatgcggtgatcgacaccaacctgacctcgctgttcaacgtcaccaagcaggtgatcgacggcatggccgaccgtggctggggccgcatcgtcaacatctcgtcggtgaacgggcagaagggccagttcggccagaccaactactccaccgccaaggccggcctgcatggcttcaccatggcactggcgcaggaagtggcgaccaagggcgtgaccgtcaacacggtctctccgggctatatcgccaccgacatggtcaaggcgatccgccaggacgtgctcgacaagatcgtcgcgacgatcccggtcaagcgcctgggcctgccggaagagatcgcctcgatctgcgcctggttgtcgtcggaggagtccggtttctcgaccggcgccgacttctcgctcaacggcggcctgcatatgggctga

SEQ ID NO: 72 - DNA, 741 bp, synthetic construct
  source 1..741: mol_type = other DNA
atgacgaaacgcatagcgtacgtgacgggcggcatgggcggcattggcacaagcatctgccagcgtctgcataaggacggctatacggtcgtcgcgggttgcgccccgaactctccgcgccgtgtcaaatggctcgaggaacagaaggcgaacggctatgacttcatcgcgtccgagggcaacgtcggcgactgggagtccaccaagaacgccttcgacaaggtgaaagccgaagtcggcgaagtcgacatcctggtgaacaacgcgggcatcacgcgcgacgtcgtgttccgcaagatgacgcacgaggactggacggccgtcatccacaccaacctgacgagcctcttcaacgtgaccaagcaggtggtccacggcatggtggagcgcggtttcgggcggatcatcaacatttcgtcggtgaacggccacaaagggcagttcggccagaccaactactctacggcgaaagccggcatccacggcttcacgatggcgctcgcgcaggaagtggcgaccaagggcgtgacggtcaacaccgtgtcgccaggctatatcggcacggacatggtcaaggcgatccgccccgaggtgctggagaagatcgtcgcgacgattccggtgcgccgtctcggccgcccggacgagatcggctcgatcgtgtcgtggctggcatcggaggaatcgggcttctcgaccggtgcggacttctcgctcaacggcgggctgcacatgggctga

SEQ ID NO: 73 - DNA, 738 bp, synthetic construct
  source 1..738: mol_type = other DNA
atgactcaaaaactcgcttacgtgacgggcggcatgggcggcatcggtacttcgatgtgccaacgcctgcacaaggacggcttcaaggtcatcgccggctgcgctccgagccgcgactaccagaagtggctggacgagcagaaggccctgggctacacgttctacgcctcggtgggcaacgtggccgactgggactccaccgtcgtcgccttcgagaaggtcaaggccgagcacggcacggtggacgtgctggtgaacaacgccggcatcacgcgtgacggccagttccgcaagatgagcaaggccgattggcaggccgtgatgtccaccaacctggacagcatgttcaacgtcaccaagcaggtgatcgacggcatgctggacaagggctggggccgcatcatcaacatctcctcggtcaacggcgagaagggccagttcggccagaccaactactccgccgccaaggccggcatgcacggcttcaccatggccctggcgcaggaagtggctgccaagggcgtgacggtcaacaccgtgagccccggctacatcgccaccgacatggtcaaggccatccgccaggacgtgctggacaagatcgtctccaccattcccatcaagcgcctgggcaccccggaggaaatcgcctccatcgtggcctggctggcgggcgacgaatccggcttcaccaccggtgccgacttcagctgcaacggcggcctgcacatgggctga

SEQ ID NO: 74 - DNA, 741 bp, synthetic construct
  source 1..741: mol_type = other DNA
atggctcgtatcgcactcgtcaccggcggcatcggcggcatcggcacttcgatctgcacacgcctggcaaaggatggctgcaccgtcgtggcgaactgcgctccgtccgaggcggccgccgccgaagagtggaagcaggcccgtgccgccgaggggttcgacatcgccgtctttaccgctgacgtgtcctcgttcgacgacagcgcgcgcatggttcgcgagatcacagagcaggtcggtcccatcgacatcctggtcaactgtgccggcatcacccgcgacaagaccttcaagaagatggagcaggcgcactgggaggccgtgatcaacgtcaacctcaacagcgtcttcaacgtcacccgtcaggtgtgggacgggatgctggagcgcggcttcgggcgtatcatcaacatctcgtcggtcaacggtcagcgcggccagttcggtcaggccaactattccgccgccaaggccggtatgcacggcttcaccatggctctggctcaggagggtgcgtccaagggcgtgaccgtcaacaccatctcgcccggctatgtcgagacggccatgaccctggcgatgaacgacgatgtgcgcaacagcatcatcagcggtattccgatgcgtcgcatggctcagcctgatgagatcgccgccgccatcgctttcctggccggcgacgagagcggttatatgacgggcgccaatctgccggtcaacggcggtctgttcatgcattga

SEQ ID NO: 75 - DNA, 744 bp, synthetic construct
  source 1..744: mol_type = other DNA
atgagcaatcaacgaattgcattcgtaacgggcggcatgggtggaatcgggacctcaatcagtcagcgcctttacaaggaaaatttcaaagtcatcgtcggatgcgccccacaatccaaacgcaaagatggctggctctccgcccagcgcgatagcggtttcagcttcgaagcctgtgaacatgacgtcaccgattgggaaagcacccagcgtgccttcgccgaactgcgcgaacgcgtcggcacaatcgatgtgctagtaaacaatgctggcattacccgcgacgccagcttccgcaagctcactccggaaaactggagtgcagtgatcaacaccaacctcaacggcatgttcaacaccaccaaacaggtcattgaagacatgctcggcaagggctggggccgcatcatcaacatctcctccatcaacggccagcgcggccagttcggccagaccaactactccgcggccaaagccggtattcatggcttcaccatggccctggcccgcgaagtggccagcaagggcgtgaccgtcaacacgatttcccctggctacatcctcaccgaaatgactggagccatgcgcccggaagttctcgaacagatcgctgccggcattccggtcggtcgccttggacagcccgaggaaatcgccagcatggttgcctggctggcctctgatgaggctgcctatgccactggcgccgacttctccatcaacggcggtctgaacatgcaatga

SEQ ID NO: 76 - DNA, 744 bp, synthetic construct
  source 1..744: mol_type = other DNA
atgacaacacgaatcgctttggtgactggcggcatgggtgggctgggcgaggccatcagcctgcgtcttgccgatgccggataccgcgttgcagtgacctgtgcccccacgaatcacgattgcgaaggctgggtcgagcgcatgcgcgagaccggtcgtgaattcgctgcctatcgtgtcgacgttgccgacttcgcgtcatgcgaggcctgcgcgagggcggtggaatccgacacggggccggtggacattctcatcaacaatgcggggatcacgcgcgacgccacgatgcgcaagatgacggccgaggactggcagtcggtattgcgcacgaatctggacagcgttttcaacatgacccgcccgctcttcgggggcatggtggcgcgtggttggggacgcatcatcaacgtcgcgtcggtcaacggcagtcgcggcgctttcgggcaggcgaactatgcggcgtcgaaggcgggcatgcacggattcaccaaatccctcgccctggaagtcgccaaatcgggggtcaccgtcaacaccatctcgccggggtacctcgcgacgaagatggtcacagcggtgccaaaggaagtgctcgaatcgcgcattcttccgcaaattccggtcggtcgcctcggacggcccgacgaggtggccgcgctcgtcgcattcctcgtatctgacgacgccgctttcatcaccggaagcaacctcgccatcaacggcggcatgcacatggagtag

SEQ ID NO: 77 - DNA, 744 bp, synthetic construct
  source 1..744: mol_type = other DNA
atgactaagcgaatcgcactggtgaccggcggcatgggcggactcggcgaggcagtcgccatcaagctgcacgacgcaggctacgcggtcgtcgtgacgcatgcgccgggcaacgcgaaggccggcgaatggctcgcgagcatggatcgccagggccgcaacttccgcgcgtatccggtcgacgtcgccgattacgattccgcccagcactgcgtcgcgaagatccaggccgaagtcggcccgatcgatatcctcgtgaacaacgccggcatcacgcaggacacgaccttcaagaagatgaccaaggtgaactgggacgcggtgctgcgcaccaatctcgattcggtcttcaacatgaccaagccggtttgcgaagagatggtgtcgcgcggctggggtcgcatcatcaacatttcgtcggtgaatggatcgaaaggccagatcggtcagacgaactattcggcggcgaaggcgggcatgcacggcttcacgaagtcgctcgcgctcgaagtcgcgaagaagggcgtgaccgtgaacacgatctcgccgggctatctcgcgaccaagatggtgaccgcgattccgcaggagattctcgacacgaagattcttccgcagattccggcgggacgtctcggcaagcccgaggaagtcgcggcgctcgtcgcgttcctgtgctcggacgatgcgggtttcgtcaccggttcgaacatcgcgatcaacggcggccagcacatgagctga

SEQ ID NO: 78 - DNA, 744 bp, synthetic construct
  source 1..744: mol_type = other DNA
atgacgcaacgtgttgctttggttacaggtgctatgggtggaatcggaacggctgtttgccaggaactggccaaggccggccacaaggtggttgccgcctacgctccggagttcgacaagccggaagagtggacaaaggccatggctgaagccggtttcaacgatttcatctgtgtcgctggcgatgtctccgactatgactcctgcgtcgctcttaccgcggaggcggaagccaaggtaggtccgatcgacattctggtcaacaatgccggcatcacacgtgacaagatgttcgcgcggatggagctggcgcagtggaatgccgtgatttcaaccaacctcaatagcctcttcaacatgaccaagcaggtctcatcgaagatggccgagcgcggctggggcaggatcatcaacatctcctcggttaatggcctccgtggccaagctggtcagaccaattactccgccgccaaagcgggcgtgattggctttaccaaggcgctggccgccgagctggccgccaagaacgtgacggtcaacgccatttgccctggctatgtagccaccccaatggtgatggcgatcaagccggaggtcctgcagagcatcatcgatacggtgccgatgaagcgtctggcgaagccggaagaaatcgggggtgcgtgtgcctaccttgcttcggacattgccggcttcatgacgggttcgacgatgaacatctgtggcggcctctactatcagtag

SEQ ID NO: 79 - protein, 393 aa, Cupriavidus necator
MTDVVIVSAARTAVGKFGGSLAKIPAPELGAVVIKAALERAGVKPEQVSEVIMGQVLTAGSGQNPARQAAIKAGLPAMVPAMTINKVCGSGLKAVMLAANAIMAGDAEIVVAGGQENMSAAPHVLPGSRDGFRMGDAKLVDTMIVDGLWDVYNQYHMGITAENVAKEYGITREAQDEFAVGSQNKAEAAQKAGKFDEEIVPVLIPQRKGDPVAFKTDEFVRQGATLDSMSGLKPAFDKAGTVTAANASGLNDGAAAVVVMSAAKAKELGLTPLATIKSYANAGVDPKVMGMGPVPASKRALSRAEWTPQDLDLMEINEAFAAQALAVHQQMGWDTSKVNVNGGAIAIGHPIGASGCRILVTLLHEMKRRDAKKGLASLCIGGGMGVALAVERK

SEQ ID NO: 80 - DNA, 1182 bp, Cupriavidus necator
  source 1..1182: mol_type = genomic DNA
atgactgacgttgtcatcgtatccgccgcccgcaccgcggtcggcaagtttggcggctcgctggccaagatcccggcaccggaactgggtgccgtggtcatcaaggccgcgctggagcgcgccggcgtcaagccggagcaggtgagcgaagtcatcatgggccaggtgctgaccgccggttcgggccagaaccccgcacgccaggccgcgatcaaggccggcctgccggcgatggtgccggccatgaccatcaacaaggtgtgcggctcgggcctgaaggccgtgatgctggccgccaacgcgatcatggcgggcgacgccgagatcgtggtggccggcggccaggaaaacatgagcgccgccccgcacgtgctgccgggctcgcgcgatggtttccgcatgggcgatgccaagctggtcgacaccatgatcgtcgacggcctgtgggacgtgtacaaccagtaccacatgggcatcaccgccgagaacgtggccaaggaatacggcatcacacgcgaggcgcaggatgagttcgccgtcggctcgcagaacaaggccgaagccgcgcagaaggccggcaagtttgacgaagagatcgtcccggtgctgatcccgcagcgcaagggcgacccggtggccttcaagaccgacgagttcgtgcgccagggcgccacgctggacagcatgtccggcctcaagcccgccttcgacaaggccggcacggtgaccgcggccaacgcctcgggcctgaacgacggcgccgccgcggtggtggtgatgtcggcggccaaggccaaggaactgggcctgaccccgctggccacgatcaagagctatgccaacgccggtgtcgatcccaaggtgatgggcatgggcccggtgccggcctccaagcgcgccctgtcgcgcgccgagtggaccccgcaagacctggacctgatggagatcaacgaggcctttgccgcgcaggcgctggcggtgcaccagcagatgggctgggacacctccaaggtcaatgtgaacggcggcgccatcgccatcggccacccgatcggcgcgtcgggctgccgtatcctggtgacgctgctgcacgagatgaagcgccgtgacgcgaagaagggcctggcctcgctgtgcatcggcggcggcatgggcgtggcgctggcagtcgagcgcaaataa

SEQ ID NO: 81 - protein, 589 aa, Cupriavidus necator
MATGKGAAASTQEGKSQPFKVTPGPFDPATWLEWSRQWQGTEGNGHAAASGIPGLDALAGVKIAPAQLGDIQQRYMKDFSALWQAMAEGKAEATGPLHDRRFAGDAWRTNLPYRFAAAFYLLNARALTELADAVEADAKTRQRIRFAISQWVDAMSPANFLATNPEAQRLLIESGGESLRAGVRNMMEDLTRGKISQTDESAFEVGRNVAVTEGAVVFENEYFQLLQYKPLTDKVHARPLLMVPPCINKYYILDLQPESSLVRHVVEQGHTVFLVSWRNPDASMAGSTWDDYIEHAAIRAIEVARDISGQDKINVLGFCVGGTIVSTALAVLAARGEHPAASVTLLTTLLDFADTGILDVFVDEGHVQLREATLGGGAGAPCALLRGLELANTFSFLRPNDLVWNYVVDNYLKGNTPVPFDLLFWNGDATNLPGPWYCWYLRHTYLQNELKVPGKLTVCGVPVDLASIDVPTYIYGSREDHIVPWTAAYASTALLANKLRFVLGASGHIAGVINPPAKNKRSHWTNDALPESPQQWLAGAIEHHGSWWPDWTAWLAGQAGAKRAAPANYGNARYRAIEPAPGRYVKAKA

SEQ ID NO: 82 - DNA, 1770 bp, Cupriavidus necator
  source 1..1770: mol_type = genomic DNA
atggcgaccggcaaaggcgcggcagcttccacgcaggaaggcaagtcccaaccattcaaggtcacgccggggccattcgatccagccacatggctggaatggtcccgccagtggcagggcactgaaggcaacggccacgcggccgcgtccggcattccgggcctggatgcgctggcaggcgtcaagatcgcgccggcgcagctgggtgatatccagcagcgctacatgaaggacttctcagcgctgtggcaggccatggccgagggcaaggccgaggccaccggtccgctgcacgaccggcgcttcgccggcgacgcatggcgcaccaacctcccatatcgcttcgctgccgcgttctacctgctcaatgcgcgcgccttgaccgagctggccgatgccgtcgaggccgatgccaagacccgccagcgcatccgcttcgcgatctcgcaatgggtcgatgcgatgtcgcccgccaacttccttgccaccaatcccgaggcgcagcgcctgctgatcgagtcgggcggcgaatcgctgcgtgccggcgtgcgcaacatgatggaagacctgacacgcggcaagatctcgcagaccgacgagagcgcgtttgaggtcggccgcaatgtcgcggtgaccgaaggcgccgtggtcttcgagaacgagtacttccagctgttgcagtacaagccgctgaccgacaaggtgcacgcgcgcccgctgctgatggtgccgccgtgcatcaacaagtactacatcctggacctgcagccggagagctcgctggtgcgccatgtggtggagcagggacatacggtgtttctggtgtcgtggcgcaatccggacgccagcatggccggcagcacctgggacgactacatcgagcacgcggccatccgcgccatcgaagtcgcgcgcgacatcagcggccaggacaagatcaacgtgctcggcttctgcgtgggcggcaccattgtctcgaccgcgctggcggtgctggccgcgcgcggcgagcacccggccgccagcgtcacgctgctgaccacgctgctggactttgccgacacgggcatcctcgacgtctttgtcgacgagggccatgtgcagttgcgcgaggccacgctgggcggcggcgccggcgcgccgtgcgcgctgctgcgcggccttgagctggccaataccttctcgttcttgcgcccgaacgacctggtgtggaactacgtggtcgacaactacctgaagggcaacacgccggtgccgttcgacctgctgttctggaacggcgacgccaccaacctgccggggccgtggtactgctggtacctgcgccacacctacctgcagaacgagctcaaggtaccgggcaagctgaccgtgtgcggcgtgccggtggacctggccagcatcgacgtgccgacctatatctacggctcgcgcgaagaccatatcgtgccgtggaccgcggcctatgcctcgaccgcgctgctggcgaacaagctgcgcttcgtgctgggtgcgtcgggccatatcgccggtgtgatcaacccgccggccaagaacaagcgcagccactggactaacgatgcgctgccggagtcgccgcagcaatggctggccggcgccatcgagcatcacggcagctggtggccggactggaccgcatggctggccgggcaggccggcgcgaaacgcgccgcgcccgccaactatggcaatgcgcgctatcgcgcaatcgaacccgcgcctgggcgatacgtcaaagccaaggcatga